European Patent Specification EP 3 665 274 B1, published October 15, 2025. Title: Variants of Family A DNA Polymerase and uses thereof. Applicant: DNAScript. The sequence listing filed with the application follows.

SEQUENCE LISTING (19 sequences)

SEQ ID NO: 1 - protein, 2590 aa, artificial sequence
  Human Pol theta
MNLLRRSGKRRRSESGSDSFSGSGGDSSASPQFLSGSVLSPPPGLGRCLKAAAAGECKPTVPDYERDKLLLANWGLPKAVLEKYHSFGVKKMFEWQAECLLLGQVLEGKNLVYSAPTSAGKTLVAELLILKRVLEMRKKALFILPFVSVAKEKKYYLQSLFQEVGIKVDGYMGSTSPSRHFSSLDIAVCTIERANGLINRLIEENKMDLLGMVVVDELHMLGDSHRGYLLELLLTKICYITRKSASCQADLASSLSNAVQIVGMSATLPNLELVASWLNAELYHTDFRPVPLLESVKVGNSIYDSSMKLVREFEPMLQVKGDEDHVVSLCYETICDNHSVLLFCPSKKWCEKLADIIAREFYNLHHQAEGLVKPSECPPVILEQKELLEVMDQLRRLPSGLDSVLQKTVPWGVAFHHAGLTFEERDIIEGAFRQGLIRVLAATSTLSSGVNLPARRVIIRTPIFGGRPLDILTYKQMVGRAGRKGVDTVGESILICKNSEKSKGIALLQGSLKPVRSCLQRREGEEVTGSMIRAILEIIVGGVASTSQDMHTYAACTFLAASMKEGKQGIQRNQESVQLGAIEACVMWLLENEFIQSTEASDGTEGKVYHPTHLGSATLSSSLSPADTLDIFADLQRAMKGFVLENDLHILYLVTPMFEDWTTIDWYRFFCLWEKLPTSMKRVAELVGVEEGFLARCVKGKVVARTERQHRQMAIHKRFFTSLVLLDLISEVPLREINQKYGCNRGQIQSLQQSAAVYAGMITVFSNRLGWHNMELLLSQFQKRLTFGIQRELCDLVRVSLLNAQRARVLYASGFHTVADLARANIVEVEVILKNAVPFKSARKAVDEEEEAVEERRNMRTIWVTGRKGLTEREAAALIVEEARMILQQDLVEMGVQWNPCALLHSSTCSLTHSESEVKEHTFISQTKSSYKKLTSKNKSNTIFSDSYIKHSPNIVQDLNKSREHTSSFNCNFQNGNQEHQTCSIFRARKRASLDINKEKPGASQNEGKTSDKKVVQTFSQKTKKAPLNFNSEKMSRSFRSWKRRKHLKRSRDSSPLKDSGACRIHLQGQTLSNPSLCEDPFTLDEKKTEFRNSGPFAKNVSLSGKEKDNKTSFPLQIKQNCSWNITLTNDNFVEHIVTGSQSKNVTCQATSVVSEKGRGVAVEAEKINEVLIQNGSKNQNVYMKHHDIHPINQYLRKQSHEQTSTITKQKNIIERQMPCEAVSSYINRDSNVTINCERIKLNTEENKPSHFQALGDDISRTVIPSEVLPSAGAFSKSEGQHENFLNISRLQEKTGTYTTNKTKNNHVSDLGLVLCDFEDSFYLDTQSEKIIQQMATENAKLGAKDTNLAAGIMQKSLVQQNSMNSFQKECHIPFPAEQHPLGATKIDHLDLKTVGTMKQSSDSHGVDILTPESPIFHSPILLEENGLFLKKNEVSVTDSQLNSFLQGYQTQETVKPVILLIPQKRTPTGVEGECLPVPETSLNMSDSLLFDSFSDDYLVKEQLPDMQMKEPLPSEVTSNHFSDSLCLQEDLIKKSNVNENQDTHQQLTCSNDESIIFSEMDSVQMVEALDNVDIFPVQEKNHTVVSPRALELSDPVLDEHHQGDQDGGDQDERAEKSKLTGTRQNHSFIWSGASFDLSPGLQRILDKVSSPLENEKLKSMTINFSSLNRKNTELNEEQEVISNLETKQVQGISFSSNNEVKSKIEMLENNANHDETSSLLPRKESNIVDDNGLIPPTPIPTSASKLTFPGILETPVNPWKTNNVLQPGESYLFGSPSDIKNHDLSPGSRNGFKDNSPISDTSFSLQLSQDGLQLTPASSSSESLSIIDVASDQNLFQTFIKEWRCKKRFSISLACEKIRSLTSSKTATIGSRFKQASSPQEIPIRDDGFPIKGCDDTLVVGLAVCWGGRDAYYFSLQKEQKHSEISASLVPPSLDPSLTLKDRMWYLQSCLRKESDKECSVVIYDFIQSYKILLLSCGISLEQSYEDPKVACWLLDPDSQEPTLHSIVTSFLPHELPLLEGMETSQGIQSLGLNAGSEHSGRYRASVESILIFNSMNQLNSLLQKENLQDVFRKVEMPSQYCLALLELNGIGFSTAECESQKHIMQAKLDAIETQAYQLAGHSFSFTSSDDIAEVLFLELKLPPNREMKNQGSKKTLGSTRRGIDNGRKLRLGRQFSTSKDVLNKLKALHPLPGLILEWRRITNAITKVVFPLQREKCLNPFLGMERIYPVSQSHTATGRITFTEPNIQNVPRDFEIKMPTLVGESPPSQAVGKGLLPMGRGKYKKGFSVNPRCQAQMEERAADRGMPFSISMRHAFVPFPGGSILAADYSQLELRILAHLSHDRRLIQVLNTGADVFRSIAAEWKMIEPESVGDDLRQQAKQICYGIIYGMGAKSLGEQMGIKENDAACYIDSFKSRYTGINQFMTETVKNCKRDGFVQTILGRRRYLPGIKDNNPYRKAHAERQAINTIVQGSAADIVKIATVNIQKQLETFHSTFKSHGHREGMLQSDQTGLSRKRKLQGMFCPIRGGFFILQLHDELLYEVAEEDVVQVAQIVKNEMESAVKLSVKLKVKVKIGASWGELKDFDV

SEQ ID NO: 2 - protein, 799 aa, artificial sequence
  pol Theta polymerase domain
GFKDNSPISDTSFSLQLSQDGLQLTPASSSSESLSIIDVASDQNLFQTFIKEWRCKKRFSISLACEKIRSLTSSKTATIGSRFKQASSPQEIPIRDDGFPIKGCDDTLVVGLAVCWGGRDAYYFSLQKEQKHSEISASLVPPSLDPSLTLKDRMWYLQSCLRKESDKECSVVIYDFIQSYKILLLSCGISLEQSYEDPKVACWLLDPDSQEPTLHSIVTSFLPHELPLLEGMETSQGIQSLGLNAGSEHSGRYRASVESILIFNSMNQLNSLLQKENLQDVFRKVEMPSQYCLALLELNGIGFSTAECESQKHIMQAKLDAIETQAYQLAGHSFSFTSSDDIAEVLFLELKLPPNREMKNQGSKKTLGSTRRGIDNGRKLRLGRQFSTSKDVLNKLKALHPLPGLILEWRRITNAITKVVFPLQREKCLNPFLGMERIYPVSQSHTATGRITFTEPNIQNVPRDFEIKMPTLVGESPPSQAVGKGLLPMGRGKYKKGFSVNPRCQAQMEERAADRGMPFSISMRHAFVPFPGGSILAADYSQLELRILAHLSHDRRLIQVLNTGADVFRSIAAEWKMIEPESVGDDLRQQAKQICYGIIYGMGAKSLGEQMGIKENDAACYIDSFKSRYTGINQFMTETVKNCKRDGFVQTILGRRRYLPGIKDNNPYRKAHAERQAINTIVQGSAADIVKIATVNIQKQLETFHSTFKSHGHREGMLQSDQTGLSRKRKLQGMFCPIRGGFFILQLHDELLYEVAEEDVVQVAQIVKNEMESAVKLSVKLKVKVKIGASWGELKDFDV

SEQ ID NO: 3 - protein, 10 aa, artificial sequence
  fragment of Pol theta
DYSQLELRIL

SEQ ID NO: 4 - protein, 8 aa, artificial sequence
  fragment of Pol Theta
PGGSILAA

SEQ ID NO: 5 - protein, 16 aa, artificial sequence
  fragment of Pol Theta
DDLRQQAKQICYGIIY

SEQ ID NO: 6 - protein, 6 aa, artificial sequence
  fragment of Pol Theta
EWRRIT

SEQ ID NO: 7 - DNA, 20 bp, artificial sequence
  primer
taatacgactcactataggg

SEQ ID NO: 8 - DNA, 19 bp, artificial sequence
  primer
gctagttattgctcagcgg

SEQ ID NO: 9 - DNA, 18 bp, artificial sequence
  primer
aaaaaaaaaaaaaagggg

SEQ ID NO: 10 - protein, 2590 aa, human; identical to SEQ ID NO: 1

SEQ ID NO: 11 - protein, 2536 aa, T. chinensis
MNLLRRSGKRRRTDSGSDSFSGSGGDSCASTVLLSKQLGCGQIPLPGEGRAPTRVQYSLQILNPGECKQTDPDDPIDKLLLANWGLPKAVLEKYHSFGVKKMFEWQAECLLLGQVLEGKNLVYSAPTSAGKTLVAELLILKRVLEMRKKALFILPFVSVAKEKKYYLQSLFQEVGIKVDGYVGSTSPTGHFSSLDIAVCTIERANGLINRLIEENKMDLLGMVVVDELHMLGDSHRGYLLELLLTKICYITQKSASCQADLVSPLFNGVQIVGMSATLPNLDLIASWLNAELYHTDFRPVPLLETVKIGNSIYDSSMKLVREFQPMLQVKGDEDHIVSLCYETICDNHSVLLFCPSKKWCEKLADTIAREFYNLHHQAEGLVKPPEFPPVTLEPKGLQEVMDQLKHLPSGLDSVLQKTVPWGVAFHHAGLTFEERDIIEGAFRQGLIRVLAATSTLSSGVNLPARRVIIRTPIFSGRPLDVLTYKQMVGRAGRKGVDTVGESILVCKISEKSKGTALLQGSLKPVCSCLRRHEGEEVTACMIRAILEIIVGGVASTPQDMQNYASCTFLAASMKEGQQEIERNQNSVQLGAIEACVMWLLENEFIQVAEVGDGTEGKVYHPTHLGSATLSSSLSPTDTLDIFADLQRAMKGFVLENDLHIVYLITPMFEDWTTIDWYRFFCLWEKLPISMKRVAELVGVEEGFLARCVKGKVVARTERQHRQMAIHKRFFTSLVLLDLISEVPLKEINQKYGCNRGQIQSLQQSAAVYAGMITVFSNRLGWHNMELLLSQFQKRLTFGIQRELCDLVRVSLLNAQRARALYASGFLTVADLARANIADVEMVLKNAVPFKSARKAVDEEEDAAEERRNMQTIWVTGRKGLTEREAAALIVEEAKMILQEDLVEMGVQWNPHSPLNSSKLSLTSSDSEVKELIFIPQTQSSCKRLISKNKSNSIFSDSYVKRSLNTVQDLDKSRERHTSPIYKFQDKNQEYQRHSISKRACLDISKEKPGTSLNEGRKSTQKAVQTFSFEKTKIASNFSSDKMSTSFRSWKHRKHLKQSRSSSSVKDSSISRTDLQRWRKSSPILCEDPSALGERNVEFRSPGPFAKNVSFCVERKYDQTEQSCTRSGAISNDIFVEHFDTGSQSKTMACQTFGVVSENGRGLAIVETEKINKVLIQNDSKNQNVNLKYCVTHPVNQDLGKQCDQQTDTCTKQKEITERQMPFEAVSSNTNGDSDVTSVKCKSVKFNSEENKPSHFQAFGNNISRTQIPSEIQVLTGTFRESGGQHDSFQNTSKIQEKACAYLTNKTENNNVSDLGLVLCDFEDSFYLDTQSEKIIQEIATENAKQAAEDPNLAAEKMQTNVQKQNLISSFQNALCVTLPGEQHSPGVTNTEPLDHKTGDTRHKPSTDSCRVDILTRENSVFHSPILLEENSPCFKGNELSVTDSQLNNFLQGYQTQETVKPGIPVVPQKETPTAMEGECLPVPETSLNMSDSLLFDSFNEDYLVKEQPAKVQAKETFLTTEITSDHFSDSLNIREGPAKTSDINGNQDIHQQLTCFNDESLMFSEMDSAQVVEVLDKLDIFPIQEKHNTAVSLSTLKLSDPVIVVNNHRQGEVIGGEQDEKAQQSKITETGQNNSFMWSGASFDLSPGLQRILDKVSSPLENEMLKSMPINLSSLKGKNRELNEKQEVISNLDTSQMQRISCFHTNEVKNNIAPENSVNHGAHLSPLSFKESCIVDDNGLIPPTPVPASASKFSFPGILGTSAVLQNTGSVLQSGGSYLFGSPSDTKNHELSPDSRNGFKDESPRKEKSFSLQFSQDGLQLTPASSNSQSLAIIDVASNQTLFQTFIKEWQCKKRFSISLACEKIGSSASSKTATIGGRFKQGSSSQETPIRDGGFPVKGHEDILVVGLAVCWGGRDAYYFSLQQEQKHSEISASLNPPPLDPGLTVKDRLWHLQSCLQKKSGKECSVIIYDFIQSYKILLLSCGISLEQDFEDPKVACWLLDPDSKEPTLHSIVTSFLPHELPLLEGMETGEGIQSLGLNVNTEHSGRYRASVESVLIFSCMTQLNSLLQKENLQDVFCKVEMPSQYCLALLELNGIGFSTAECESQKQIMQAKLDAIETEAYQLAGHSFSFTSSDDIAEVLFLELKLPPNGEMKNQGIKKTLGSTRRGIDSGRKLRLGRQFSTRRITFTEPNIQNVPRDFEIKMPTLVEESPPSQALGKGLLPMGRGKIKKGRRLNPEHQAHLEERASDKGMPFSVSMRHAFVPFPGGLILAADYSQLELRILAHLSHDHRLIQVLNTGADVFRSIAAEWKMIEPETVGNELRQQAKQICYGIIYGMGAKSLGEQMGIKENDAACYIDSFKSRYTGINHFMRETVKNCKRDGFVQTILGRRRYLPGIKDNNPYHKAHAERQAINTTVQGSAADIVKVATVNIQKQLETLRSTFKSHGHRESMLRRDKTGLLPKRKLQGMFCPIRGGFFILQLHDELLYEVAEEDAVQVAQIVKNEMENAIKLSVKLKVKVKIGASWAELRDFDV

SEQ ID NO: 12 - protein, 2383 aa, C. griseus
MRKKALFILPFVSVAKEKKYYLQSLFQEVGIKVDGYMGSSSPTGRFSSLDIAVCTIERANGLINRLIEENKMDLLGMVVVDELHMLGDSHRGYLLELLLTKICYVTRKSTLCQADSARALCNAVQIVGMSATLPNLQLVASWLDAELYHTDFRPVPLLESIKIGNSIYDSSMKLVRELQPVLQVKGDEDHIVSLCYETVCDNHSVLLFCPSKKWCEKVADIIAREFYNLHHQPERLVKPSEFPPVNLDQKSLLEVMDQLKRSPSGLDSVLKNTVPWGVAFHHAGLTFEERDIIEGAFRQGLIRVLAATSTLSSGVNLPARRVIIRTPVFGGQTLDILTYKQMVGRAGRKGVDTMAAVYDDFQIIVGGVASTSQDMQTYASCTFLAAAVKEGKQGIQRNQDDVHFGAIDACVTWLLENEFIQEAEPSDGSGGKVYHPTHLGSATLSSSLSPTDTLDIFADLQRAMKGFVLENDLHIVYLVTPVFEDWTGIDWYRFFCLWEKLPTSMKRVAELVGVEEGFLARCVKGKVVARTDRQHRQMAIHKRFFTSLVLLDLISEIPLKEINQKYGCNRGQIQSLQQSAAVYAGMITVFSNRLGWHNMELLLSQFQKRLTFGIQRELCDLIRVSLLNAQRARFLYASGFLTVADLARANVAEVEVVLKNAVPFKSTRKAVDEEEEAAEERRNMQTIWVSGRKGLSAREAATLIVEEAKTILQQDLLEMGVQWDPNSSLSSSTSSLTSSESEVNERTLQSQTKNSHKRLTSKNRNSMRASVSNDKPSPDTAQGLGEHSEHTDSLCLLQGNKHQHQPHSVCRARKRTSLGINKEKLRMSLNGGEPSTKEVLQTFSMEKTRKAALTANSEQTNTSFPSWRDRKHRKKSWGSSPVRDSRANHHRDDFQEHTVSRSTLCEEPLSLDKQNIEFRSSGLLIKNASFCANEKYNKTSFSLQMQQPCLRKKTESTGAVEHSFAESQSKNVTGQSPGVASNGRELADTETGKINEVLIENGAESQNVSVKHHDTHPISQCLENQCDKQTNTCTKRKALIERQVSCEAVSYMARDSNDVSTINSESIKLHSKDDESNHCQVLGNNTGRSEAPRGLLQSAAEFSQADGQHEHLLNSSGIQEKTDAYATNKTEHNHVSNLAPCDFGDSFYLDTQSEKIIEQLATEHAKQRTKAVTAKGSDTRNSGSSFQNKCHSTRGEQHFQRAANTDHLDSKSVETTKQNPEKSIGRLTAESIIFHSPTPQGENGPCFRVNEQSVTDSQLNSFLQGFETQEMVKPVLSLAPLAGTPTGLEEENLPETSLNMSDSILFDSFGEDDLVKGQSPDVQAKQPLLSVMTPNHLSSSLCPREDPVMKANVNDHQGIQQPETCSSGESVIFSEVDSAQMIEALDSVAALHVQQNCNSVTLKTLELSDSAMLDNECPQGKVARGDKSERAQMSKLTETNQDNSITWSGASFDLSPELQRILDKGSSPLENERPKLTQTNLSCFERNGTELNERQEMNPNLEAVQIQRTSLFPNNGVQNKIEGIGNDTRRGEALYPSARKESDTADDNGLIPPTPILASTSKLSFPEILGTSVNHLKADSVFLPGESCLFGSPSDSQERRDSFKDDRSVGDTSFSLQFSQDELQLTPASCSSESLAIIDVASDHTLFETFVKEWRCQKRFSISLACEKIRSPTSSKTATIGGRLKQVSSPQKTSAEDDGFPVHGSDGVIVVGLAVCWGGRDAYYLSLQKEQKHSVFPLRLLLQLNEFNFYIKTVLFQEISPSLAPPPLDTTLTVEERMEHLQSCLQKKSDKEQTVVTYDFIQSYKILLLSCGVSLEPSYEDPKVACWLLDPDSKEPTLHSIVTSFLPEELPLLEGIETGQGIQSLGLNVDTEHSGRYRASVESILIFNSMNQLNSLLQKENLHDIFCKVEMPSQYCLALLELNGIGFSTAECESQKHIMQAKLDAIETQAYQLAGHSFSFTSADDIAQDVLNKLKALHPLPGLILEWRRISNAITKVVFPLQREKRLNPFLRMERLYPVSQSHTATGRITFIEPNIQNVPRDFEIKMPTVVRESPPSQAPGKRLLPMTRGQNKKFYGLHPGNGTLMEEKASDRGVPFSVSMRHAFVPFPVDNLLELRILAHLSRDCRLIQVLNTGADVFRSIAAEWKMIEPDSVGEDLRQQAKQICYGIIYGMGAKSLGEQMGIKENDAACYIDSFKSRYTGINHFLRDTVKKCRRDGFVQTILGRRRYLPGIKDNNPYHKAHAERQAINTTVQGSAADIVKTATVNIQKQLETFHSAFKSHGHRESMLQHGQTGCGDLSPSPGQLVGLLPKKKLKGMFCPMRGGFFILQLHDELLYEVAEEDVVQVAQIVKKEMECAVKLSVKLKVKVRMGASWGQLEDFDV

SEQ ID NO: 13 - protein, 2530 aa, R. norvegicus
MSLPRRSGKRRRSSSGSDSFSFSGDGDSCVSPQLLCRPVLSPPPGLGRGRRLAGTGTCKQRVSDDQIDQLLLANWGLPKAVLEKYHNFGVKKMFEWQAECLLLGQVLEGKNLVYSAPTSAGKTLVAELLILKRVLETRKKALFILPFVSVAKEKKYYLQSLFQEVGIKVDGYMGSTSPTGRFSSLDVAVCTIERANGLINRLIEENKMDLLGTVVVDELHMLGDSHRGYLLELLLTKVCFVTRKSASCQADSASALACAVQIVGMSATLPNLQLVASWLNAELYHTDFRPVPLLESIKVGNSIYDSSMKLVREFQPLLQVKGDEDHIVSLCYETVRDNHSVLVFCPSKKWCEKVADIIAREFYNLHHQPEGLVKSSEFPPVILDQKSLLEVIDQLKRSPSGLDSVLKNTVPWGVAFHHAGLTFEERDIIEGAFRQGLIRVLAATSTLSSGVNLPARRVIIRTPVFGGQPLDILTYKQMVGRAGRKGVDTMGESILVCKNSEKSKGIALLQGSLEPVHSCLQSQGEVTSTMIRAILEIIVSGVASTSQDMQTYAACTFLAADVKEGKQGIQRNRDDVQRGAVDACVTWLLENEFIQAAEPSDGTGGKVYHPTHLGSATLSSSLSPTDTLDIFADLQRAMKGFVLENDLHIVYLVTPVFEDWTSIDWYRFFCLWEKLPTSMKRVAELVGVEEGFLARCVKGKVVARTERQHRQMAIHKRFFTSLVLLDLISEIPLKEINQKYGCNRGQIQSLQQSAAVYAGMITVFSNRLGWHNMELLLSQFQKRLTFGIQRELCDLIRVSSLNAQRARFLYASGFLTVADLARADTVEVEAALKDALPFKSARKAVDEEEEAAEERRSMRTIWVAGKSLSAREAAALIVEEAKVILQQDLIEMGVQWGPHSPLSSSTHSLTSGSEVKEHTFKSQTKSSHKRLASKSRNSMRVSGSNGKQSPEAGQGLDECRERPDSLCKFQGNHEIQTPSVYRARKRTSLGVNKEMLRTSLKEGKPSTKEVLQTLSFEKTRKAALSFSSEQANNSFPSGRDRKYRKKSWGSSPMSDSVMHRDDLQGQTMCKSTLCEDPQKSLEEQNTEYRSPGLFAKNVSFCAKEKCNKTSFPLQMQQPCLRRKPESGAAVDHSVAVSQNKNVVEQPPGAPRDRRGLAAHGRAEVNEVLTENGTESQLHDTHPVSQCLENHSEKQTNTCTRQKTLTEGQAGISHVTRGSNDLTPIRCERLKLNSKEHDSNPCPQALGTNAGRTEAPQSSEALGQAGGQCENLLNSPGIQEKTSAHATNKTEHSHVANQAFCDFGDSLYLDTQSEEIIEQMATKNATQGAEAAGITEEGSATQNEPHSTTGGQHIPGAANTDHVDRKNTESVKENPEKNIDRRTPHSLIFHSPTPQGGNSACFKENEHSVTDSQLNSFLQGLETQDKPIIPLAPQMRTSTGVEEESLPETSLNMSDSILFDSFGEDSFGQRQSLDVKAKQPLLSEMTPNHFHNPPYPQEDPVMTPHMSEPQGTLERMACLSGESIIFSEIDSAQVIEALDNMAAFYMQENCNPITLKTEPRDLAALGNECPQGEVVRGEQHEGSSKPKFMEINQDNSFTWSAASFNLSPELQRILDKVSTPRENEEPELMHADLSCFEENSTESHERQDMNSDLGTVQRTSFLPSNGVKSRTEGLESKAKHGGASSALPHKAAADDNGLIPPTPLPASASASASKLALPEILGTSVKHQKASCLFDSPSDNQNQDLSQELRDSLKDSDGSVVDTSFFLQSQDGLLLTQASCSSESLAIIDVASDQILFQTFVKEWQCQKRFSISLACEKMTSSTSSKTATIGGRLKQVNSPQEASVEDDGFPVHGSDCAVVVGLAVCWGGKDAYYLSLQKEQKQSEMSPSLAPPPLDATLTVKERMEYLQSCLQKKSDQERSVVTYDFIQTYKVLLLSCGISLEPSYEDPKVACWLLDPDSKEPTLHSIVTSFLPHELALLEGIETGPGIQSLGLNVNTDHSGRYRASVESVLIFNSMNQLNSMLQKENLHDIFCKVEMPSQYCLALLELNGIGFSTAECETQKHIMQAKLDAIETQAYQLAGHSFSFTSADDIAQVLFLELKLPPNGEMKTQGGRKTLGSTRRGTESDRKLRLGRRFSTSKDILNKLKDLHPLPGLILEWRRISNAITKVVFPLQREKHLNPFLRMERIYPVSQSHTATGRITFTEPNIQNVPRDFEIKMPTLVRESPPSQASGKGQLAMARQNQKVYGLHPGQRTVLEKTSDRGVPFSVSMRHAFVPFPGGLILAADYSQLELRILAHLSRDCRLIQVLNSGADVFRSIAAEWKMIEPDAVGDNLRQQAKQICYGIIYGMGAKSLGEQMGIKENDAACYIDSFKSRYKGINHFMRDTVKNCRRDGFVETILGRRRYLPGIKDNNPYHKAHAERQAINTTVQGSAADIVKVATVNIQKQLETFHPTFKSHGHRESMLQSDRAGLLPKRKVKGMFCPMRGGFFILQLHDELLYEVAEEDVVQVAQIVKNEMECAIKLSVKLK

SEQ ID NO: 14 - protein, 2577 aa, A. sinensis
MAFFSKGQCQRMNIPEDQADKLLLASWGLPKAVLEKYHSLGVVHMFKWQAECLMLGQVLEGKNLVYSAPTSAGKTLVAELLILKRVLETHKKALFILPFVSVAKEKKYYLQALFQEVGVRVEGYMGSTSPAGRFSTLDVAVCTIERANGLINRLIEENQMDLLGMVVVDELHMLGDSHRGYLLELLLTKVRFITEKVTKRQAKASSPAFGGIQIVGMSATLPNLHLLASWLNAELYHTDFRPVPLMEWVKIGSNIYDSSMNLVREFQPMLQLKGDEDHVVSLCYETVRDGHSVLLFCPSKNWCEKLANIIAREFCNLQLSDRKTSNLPPIPLYKEAIEEVMDQLRRSLSGLDSVLQRTLPWGVAFHHAGLTFDERDVIEGAFRQGLIRVLAATSTLSSGVNLPARRVIIRTPVFGGKLLDILAYKQMAGRAGRKGADTVGESILVCKPSERSKGIALLQGSLKPVRSCLLRREGEGITSSMIRAILEIIVGGVASTPDDVRTYASCTLLVASLKDNEQGSEKNEDGVQNGAIEACVAWLLQNEFIQVSGPSDGVKAEVYCPTHLGSATLSSSLSPMEALEIFADLQRAMKGFVLENDLHIVYLVTPVYEEWTTIDWYQFFCLWEKLPASMKRVAELVGIEEGFLARSVKGKIIAKTEKQHRQMAIHKRFFTSLALLDLISEVPLKDITKRYGCSRGQLQSLQQSAATYAGMVTVFSNRLGWHNMEQLLSQFQSRLTFGVHRELCDLVRVSLLNAQRARALYNTGFITVADLAKANPADVETALKTTVPFKSLRRAVDEDEEAAEERRNARCIWMAGMKHVTENEAASLVVEEARMLLQQDLAVMGVQWNPDSYLDSESSSSMISSESELEDRKYRLSREGSFETLKAFNKERYGLHPNSQSGTSAKIEKGNKRLLGASTPKGRLQSEAQIDQIQTEEGNIDVIVQSARKRPHLSKDKENMEFTSKRKSKAGFRETSQESPTEEGKRPTLSFVPTKTSAVCRPRRIMGGSLNQSRNCSRALKQHRSLLEESRRQITGIKGPPLSRHSSSESKSFPDGSNKELTEKGSLVHKDKISGSFHEHYPLIGSKEKMEGLLMEPSVTNECKPKEKTICQASRDVIMRDAATVRMETSDTVGGLMIPSRELKNENIGAKDSKVHAGKKYAKRISGKQQMILDTDLCNEIVSSSAKTHVSDGAYKQKTVCYEPKSCLFPIQSKSKHSSESPNGVLFKSGGVGKAADNQPEDFLRDSIIKSRAVCIAKSSKNGYAHDLSLGYGYFEDSFQLDTQTDRIIQQQVASEIAGHQGAKGTELAAIAVQKTFTKLPCDNAFQTESVADKNLVAAFREMDSSGLVTTLGMKQPTDLCCSDKTLGSVSSCLQSAVKFPDAALCLRGNDFSVTDSQLHSFLQGYLTQPSVKESVCLGLQNGAPVSNGQNPHIIHVQVECHPIPETSLNTSNSLLFEDSFSDLNDPSGIRAGEAEGVETREQEILPFPPNTISSSLVGCLHQQSWGPIQDVWSINQVEEQQPPQCNDASLTFSEIDSFQLAEAFDNVSSPPFQGDLPSAALVEPELRKSVAQEDSGPMDIKGDKSVRPQKAQQNVKKNPNSIVWSEHSFELSPGLQEILDKWPSPSGNKPASSSPSIPGSKEKLVLSNCSQEQGAVFEFGCGQKKPLPLCQGLENYFTGRESNRGALEQKPNCSPKFLKGSSRKRDPQPDISNGLIPPTPPMEPAPKSFGMSSLKSGKKKDVILMNEGPLCQVLQNGIPVSDQQIETLQFNPENGDPLEIDPVKEDSVIDQDFSLQLSQDILPLISCSAESFTIIDVASDMALFQTFIQEWRNKNRFAISVACERTKRLLSSRSTIGGRFKQVRSPQQIQVKDDGFPIKGCEDTLIVGLAVCWGGKDAYYVSLQQKADDQAEVSASLAPPALDQNLSVTERLCHLQSCLQKEPEGKHCLVMYDFIQHYKTLLMACGISLEGSFEDPKVACWLLDPGSKERTLHNMVTSFLPHELPLLEGIGTGQGVQSLGLSASADHSGRYRAAVESVLIFGIMNQLNTLLQKENLTDAFCKVEMPTQYCLALLELNGIGFSTVACETQKHIMQAKLNEIETQAYQLAGHSFSLTSPDDIAEVLFLELKLPNGDVKAQGNKKTLGYTRRCTTKGHRIRLGKQFSTTKDALEKLKTLHPLPGLILEWRRITNAVTKVVFPLQREKRLNSLLGMERIYPISQTHTATGRISFAEPNIQNVPKDFEIEMPTLVEESPPSQARRNVSALPGARSRKHHSILPQGSNSVAEEGPKGRGMPFSVSMRHAFVPFPGGLILAADYSQIELRILAHLSGDRRLIQALNSGADVFKSIAAEWKMIDPEAVRDDTRQQAKQICYGIIYGIGAKSLGEQMGVEENDAASYIDSFKSRYKGIQKFLRETVNNCSRDGFVKTILGRRRYLPAIRDPNPYSKAHAERQAVNTTVQGSAADLVKTATVNIQRRLEAFPSTIKSHGHLESSFQMDRAGRLERRRNRRMLHPITGGFFILQLHDELLYEVAEDDVIQVAQIVKHEMENAMKLSVKLNVKVRIGPSWGDLQDLEL

SEQ ID NO: 15 - protein, 2596 aa, P. troglodytes
MNLLRRSGKRRRSESGSDSFSGSGGDSSDSPQLLSGSVLSPPPGLGRCLKDRGRQSAAAAGECKPTVPDYEIDKLLLANWGLPKAVLEKYHSFGVKKMFEWQAECLLLGQVLEGKNLVYSAPTSAGKTLVAELLILKRVLEMRKKALFILPFVSVAKEKKYYLQSLFQEVGIKVDGYMGSTSPSRHFSSLDIAVCTIERANGLINRLIEENKMDLLGMVVVDELHMLGDSHRGYLLELLLTKICYITRKSASCQADLASSLSNAVQIVGMSATLPNLELVASWLNAELYHTDFRPVPLLESVKVGNSIYDSSMKLVREFEPMLQVKGDEDHVVSLCYETIRDNHSVLLFCPSKKWCEKLADIIAREFYNLHHQAEGLVKPSECPPVILEQKELLEVMDQLRRLPSGLDSVLQKTVPWGVAFHHAGLTFEERDIIEGAFRQGLIRVLAATSTLSSGVNLPARRVIIRTPIFGGRPLDILTYKQMVGRAGRKGVDTVGESILICKNSEKSKGIALLQGSLKPVRSCLQRREGEEVTASMIRAILEIIVGGVASTSQDMHTYAACTFLAASMKEGKQGIQRNQESVQLGAIEACVMWLLENEFIQSTEASDGTEGKVYHPTHLGSATLSSSLSPADTLDIFADLQRAMKGFVLENDLHILYLVTPMFEDWTTIDWYRFFCLWEKLPTSMKRVAELVGVEEGFLARCVKGKVVARTERQHRQMAIHKRFFTSLVLLDLISEVPLREINQKYGCNRGQIQSLQQSAAVYAGMITVFSNRLGWHNMELLLSQFQKRLTFGIQRELCDLVRVSLLNAQRARVLYASGFHTVADLARANIVEVEVILKNAVPFKSARKAVDEEEEAVEERRNMRTIWVTGRKGLTEREAAALIVEEARMILQQDLVEMGVQWNPCALLHSSTCSLTHSESEVKEHTFISQTKSSYKKLTSKNKSNTIFSDSYIKHSPNIVQDLNKSREHTSSFNCNFQNGNQEHQRCSIFRARKRASLDINKEKPGASQNEGETSDKKVVQTFSRKTKKAPLNFNSEKMSRSFRSWKHRKHLKRSRDSSPLKDSGACRIHLQGQTLSNPSLCEDPFTLDEKKTEFRNSGPFAKNVSLSGKEKDNKTSFPLQIKQNCSWNITLTNDNFVEHIVTGSQSKNVTCQATSVVSEKGRGVAVEAEKINEVLIQNGSKNQNVYIKHHDIHPINQYLRKQSHEQTSTITKQKNIIERQMPCEAVSSYINRDSNVTINCERIKLNTEENKPSHFQALGDDISRTVIPSEVLPSAGAFSKSEGQHENFLNISRLQEKTGTYTTNKTKNNHVSDLGLVLCDFEDSFYLDTQSEKIIQQMATENAKLGAKDTNLAAGIMQKSLVQQNSMNSFQKECHIPFPAEQHPLGATKIDHLDLKTVGTMKQSTDSHGVDILTPESPIFHSPILLEENGLFLKKNEVSVTDSQLNSFLQGYQTQETVKPVIPLIPQKRTPTGVEGECLPVPETSLNMSDSLLFDSFSDDYLVKEQLPDMQMKEPLPSEVTSNHFSDSLCLQEDLIRKSNVNENQDTHQQLTCSNDESIIFSEMDSVQMVEALDNADIFPVQEKNHTVVSPRALELSDPVLDEHHQGDQDGGDQDERAEKSKLTGTRQNHSFIWSGASFDLSPGLQRILDKVSSPLENEKLKSMTINFSSLNRKNTELNEEQEVISNLETKQVQGISFSSNNEVKSKIEMLENNANHDETSSLLPRKESNIVDDNGLIPPTPIPTSASKLTFPGILETPVNPWKTNNVLQPGESYLFGSPSDIKNHDLSPGSRNGFKDNSPISDTSFSLQLSQDGLQLTPASSSSESLAIIDVASDQNLFQTFIKEWRCKKRFSISLACEKIRSLTSSKTATIGSRFKQASSPQEIPIRDDGFPIKGCDDILVVGLAVCWGGRDAYYFSLQKEQKHSEISASLVPPSLDPSLTLKDRMWYLQSCLRKESDKECSVVIYDFIQSYKILLLSCGISLEQSYEDPKVACWLLDPDSQEPTLHSIVTSFLPHELPLLEGMETSQGIQSLGLNAGSEHSGRYRASVESILIFNSMNQLNSLLQKENLQDVFRKVEMPSQYCLALLELNGIGFSTAECESQKHIMQAKLDAIETQAYQLAGHSFSFTSSDDIAEVLFLELKLPPNREMKNQGSKKTLGSTRRGIDNGRKLRLGRQFSTSKDVLNKLKALHPLPGLILEWRRITNAITKVVFPLQREKRLNPFLGMERIYPVSQSHTATGRITFIEPNIQNVPRDFEIKMPTLVGESPPSQAVGKGLLPMGRGKYKKGFSVNPRCQAQMEERAADRGMPFSISMRHAFVPFPGGSILAADYSQLELRILAHLSHDRRLIQVLNTGADVFRSIAAEWKMIEPESVGDDLRQQAKQICYGIIYGMGAKSLGEQMGIKENDAACYIDSFKSRYTGINQFMTETVKNCKRDGFVQTILGRRRYLPGIKDNNPYRKAHAERQAINTIVQGSAADIVKIATVNIQKQLETFHSTFKSHGHREGMLQSDRTGLSRKRKLQGMFCPIRGGFFILQLHDELLYEVAEEDVVQVAQIVKNEMESAVKLSVKLKVKVKIGASWGELKDFDV

SEQ ID NO: 16 - protein, 2665 aa, F. heteroclitus
MRPWQQPRDPGVCHVGEENARMASGPLKKKSYLGQHQIKKKTSIPAGDHEPTDGDGLLQKPSDKTNRAQSSGRDGLMGGRGALLPLGESTLALDEEMLQTLDAADLSKGDVKRDGKGAFPPPRPAPQTARLKLDGKPAKVDGESLPFTNGAEDPQQGGCKPRWDSNKPGWRADCKDLAQKLLFSEDSGEADRCTRNQENNRSDDAPASASALPCKETRSRQKAGGSRKQELRGRGSPPSDGKDKSMKNTDPPLDVSTDYILFSPTRLAEARRRAKLQQSLHNQSVSVLTVPSGLELSTLSDTLPPPGVAVRAPERQAEKLLLSSWGLPKPVLERYQNHGVTRMFEWQAQCLAVGQALRGGNLVYSAPTSAGKTLVSELLILKRVLETRRKALFILPFVSVAKEKMHYLQSVFEEAGIRVEGYMGSTSAAGGFTTLDVAVCTIEKANSLINRLIEENSMDLLGVVVVDELHMVGDSGRGYLLELLLTKIRYIAQKQNTSGSLAEGVQIIGMSATLPNLSLLAGWLGADLYQTDYRPVPLQEHLKVGGNIYDRSLSVVRQFTPALNVKGDDDHIVSLCYETVREGHSVLLFCPSKNWCEKLADTIARAFFNLRNTDPQSEGVPPPVCLDTAGLVDVIAQLRRTPAGLDPILQRTVPWGVGFHHAGLTFDERDVLEGAFRQGLVRVLAATSTLSSGVNLPARRVVIRTPVFNGRLLDPLTYKQMAGRAGRKGVDTTGESVLVCKQSEHQKGISLLQGALQPISSCLVRREGEGVTTSMLRAILEVIVGGVASSPRDVRLYASCSLLAASTKGDGGKESTEETSSGAIEACVDWLMGNEFISIQRDGQDEQYCPTQLGAATLSSSLSPPEALGIFADLQRAMKGFVLESDLHILYLITPLYAEWTTIDWYQFFCLWEQLPSSMKRVAELVGVQEGFLARSVSGKIVAKTEKQLRQMAVHKRFFTTLVLQDLVSEVPLGAVASKYNCNRGQLQSLQQSASTYAGMVTVFCKRLGWHNMELLLSQYQTRLSFGVQRELVDLVRLSLLNATRARALYAQGLCTVAQVARAPVADVEKALRNAVPFKSSKRAVDESEMEAAERRNLRCVWVTGGRALTEQEAAAEIVSEARLLLQEDLAQLGVHWDPSTLPPQAPSGSSSDDSHSGDSDAASAPRVAPRRSPMRRTEGHPSGTHTGRRNVSKSRGEEIGRDAEIQEKVAYGKGALEGEARKPDVTDPEISDVLVERAEGRNEAKPSTSRQDEAEHVEDKQETAGAVQHGGRLESISLVEEDRRKRNKSVEEQTHHYLNQPAVEMSLTQELAEIVSSPLPPPPPQPQPPPSPAPPPRFRAPVSRLAHRPSAPTSTGKGGCSTSPLLPRTPKHSAALRKVLQSIQTGRGVQDRLQPADLSPSKVPNAAPVTLQENPDVASTPPGADSAPLFTPEAKRRRTEAGGVDRFSSPELYAGSKTDEEEQGDAEEEEEEESFGRSLDLDTQTERMIAQRPLTGTAGGRDEAGEQQGERRGDRVKGPDDDRRDEAEGPETAAARFQISVTESQMELILNSNPRASPSPARGDTDQAGDDRQLSDNNEAAAESPDGSSGFLFDSMHDSALLDTLLLNPSPEPAGEEEEPAGPAPAPSAQQKRRSELLANQEAEEQEAVRWGESFFCLSEWGESFLVGEAFLGRQALSRHAEGGEGNQGLQQPSKEEESEEEKAGGRQRDEEKDAKHVEKLTGEERENLIENDVLKTPGVQNSPESAFYCSPGLQEIFDRWPSMSDQPGPTADTADATELPRPATQPGRKRKQPQRPDATQKAQPPERPGSAGDLIPPTQETAPVTPRVKLTTSSVLSPAVTQPLKQSTPSHRLQEGPTDGERATAHAAVSVSDRRPQRSPPTGRSLFFPPQTAASPPSPRPEPPSDAESPVSPGGFALQLSQDASLLCSDSGSFSIIDVASDRRLFDTFIKEWETKERFSVALACERRAHRRRPEDDTGGRRKRASAAHPTPDGFPVGDDEGRTLIGLSVCWGARDAYYVSLQQEQSEGLSSSLAPPPLDKALPVTQRLQRVKACLSAAPSGRRGRAVVVYDIIKVYKRLVRSCGISLEGNYEDPKVACWLLDPGREERTLPNMVTVYCPEELPLVDGLGNAHSHCPRVRAATESVLVHAVMQHLSGLLERDGALDVFRRTEMPSQVCLALLELNGVGFSAEECERQKHVMQAKLSALEAEAYSLAGHSFSLTSVDDVAQVLFLELHLPPNGDVDGPRSKKTLGYTRRGGGRARLGKQFSTTKDVLEKLRPLHPLPGVILEWRRITNALTKVVFPLQREKRYEPTLDMDRIYPVAQTHTATGRVSFTEPNIQNVPKDFEISLPTVVGESPPSQGGFQMPNRPGRRRSVAPLPAAADQGPAFSVSMRHAFVPFSGGMILAADYSQLELRVLAHLSKDQRLLQVLNGGADVFRCIAAEWKSVEPASVQDDLRQQAKQICYGIIYGMGAKSLGEQMGVEENDAACYIESFKARYKGINAFLKQTVKKCLKDGYVQTLMGRRRYLAGIANANPHVKAHAERQAVNTTVQGSAADIVKLATVNIQKRLRETYPSAPLSHQHAHSAHNNQRRFGTSRLRGAYFILQLHDELIYETTERDLIQVAQIVKREMESAVKLYVKLKAKVKVGPSWGNLQDLDI

SEQ ID NO: 17 - protein, 2674 aa, C. gigas
MTSKSKNGGMELDASFSSSFCTELDAQMLVAMETMEKQPRSQKSLPKGTKKNSPVLTSTPQSVTPLPRRQAQLMKSLFTLQSPLNDSLFSPFSSQTTDNVKDGEQLTPSSAMNGKPCRKRTRKVLNEIINEKERIDEDNGDKLLLKNWGLPEPVMKQYSDKGITSMFEWQAECLCLPGVLDGGNLVYSAPTSAGKTMVAELLVLKRVLETKKKAIIILPFVSVAREKMFYLQQLYQEVGVSVSGFMGSYSPPGGLSQVDVAVCTIEKGNGLINRLMEENRLDQLGIVVIDELHLVGDQHRGYLLELMLTKIRFLSQRMKKPDPQNMESSSTEGIQIIGMSATLPNLDLLARWLDATLYRTDYRPVPLTECVKLGADIFDSRLQKIREVDLSVTFKGDTDHVVPLCLETLRDGHSVLIFCPTKNWCEKLAETIAREFYGILKKAPVDMQANQGSGGNPPSPCLPLSRASLQEVVEQLRRTPVGLDSTLGKTVPYGVAYHHAGKYQHKFIVRVKEDPGGARLYPEEDCPYVVAHHHTGLTFDERDILEGAFRQGAVKVLIATSTLSSGVNLPARRVIIRTPLFHGKTIDFLTYKQMIGRAGRKGVDTQGESILICKPGERSKAVTLVQSALPPVSSCLIKNQGEQLSSSMKRAILEIVVSGVADSVTDVTAYASCTMLAASLDTSSDQTQGMISACIQFLQENEFVSLQRVQSSDGVYEDRFVPTQLGAAVLASSLSPDEGLSVFAELQKARQCFVLENELHIVYLVTPIYSLDLGAGMNWYKFYCLWDKLSPDKKRVAQLVGVSEAFLTRAIQGRIPTKTENQIRSLAIHKRFYTSLILSDLVQEVPLGEVCHRYGANKGQLQSLQQTAATFAGMVTVFCARLGWYNLELILGQFQHRLTFGIQRELCDLVRLTLLNGQRARVLYDGGFHTVAALANASVSDVEKIFKKSSPFQSSKKLENETEWEAARRQESRCIWLTGRKGATEREAAQAIIQEAKSLIQQELGGLGIQWKTPDTRKSLEEGSNPDQNGMDCSRDLEKSSNNHQIGLMKMKSKGSVRKRRSLSRKSPALSQARSSRGKGFNRQEKSVVISPPSFNSQSRRNKSNIGTDSGSGKPCDNDCIVIVDDSSGDPNERQGNKEIPSIKDFVVRQIEEQSCQQRNRNNPEKRDCEKNCTSEVRVQPNHMYHKDQLQIDLVKTNANCNEEAGKQLTGLHEAREKPRVEAIKANPSRCTERENVSASSSSSSSSSTSSSVINSSSRPAEDSHVFKSPIFSSVSTGIKKSGPKTRSSSFPLSTLSTSSTSLGSSTASVVMSPQLAKNKNDLIKIPSNKRNAMPNQSIQRGILSGVQQIITNSTDLETVNGKLNEHESDVRTINERRQKADLTPEANFRELRDRGDSEERKKLQEIKVNKTIEPMICSEDFADSFVFESQMDGNMEAFPGLCNEVSQSLQSKKTLGDSEKINSKIVVDKIIEKQINSNGFFQPNGSSSSKKHLVRNAHIVVEKHRTNTALSTADAATVNKEQVDDEHSTDGNDMNLSCSLLSSHDVSCDLLPASNFEKCMVSDDESDVCRDESYRDLRIPYLSGQEAACFDGNERKADLALGGYQISQGLLQELDETFSEECSQGSKGQSQRSAGQGGSFKNGKKQNNNSIDGMEASKVEQGKATEQNLKTFEKKKNGQIIERKMEEAEVGVTEEMDDSLTLSMVYEVIENCDKGQCNKNLNSKTDKSNTNQLTSRRSSQRNAKSNSKKTNEIICEELISKKSSECNKRSTLKSKESSFTKVKCSRSSQDKDKRLSPGTLAFLDDLHTSLDTDSDTIVMKTPLCQRRRGNNNKEGSTRDSVVMDEVMDEDLQNEYSGEDNVRTNECLSPTPPRLSLVNSPKTIRKATPNRHRPQKQDDRRSARKNIESLGVSMKNSKVPFVESAKSAEEEVREWNSGKLESPTGEDPPYVERGPVVDPNETGIPPSQGAFTIIDVCADKVLFDTFIKEWNCQPSFAISLACINKPRDPVTTTGGIGAKFTEAGDTGHKSSKVKTTEPGVASRGIPVWGVNLVITGVAVSWGDRDAYFITLTSENIEDEEDTDLSPPDLDKSLSVTARLAAIRQVLERKDSFTVIAMDAKACYGALERSCGICCQGEFQDPKVATWLLDPGAKEKNLHRMVHDYLPLEAFLLEDIGGGVGYGSIGMSPENPGSSRVRSCTEAVLLTHLMQFYTLCFNDEECERQKNIMVARLGDLEEQAYRCVGHQFSLTSTEDLSQILFIELQLPVNGDPSSLGQPMRPNRRAPNSHRGRQKSQFSTTKEVLEKLRPLHPFPGILLEWRRISGSLTKVVFALQKEKVYCENLGMHRIFTDVQYFTATGRVSLSEPNLQNVPKDFLISVSAPVENFNQWDAAGHRNKNRNSGQTSFNVSMRHAFIPFPGGVLLAADYSQLELRMIAHLSQDSKLIKILNGDGDVFKLITAQWKSISVEEVTPEQRQQAKQICYGMIYGIGAKALGDTLGVEENDAAAFIQTFKSKYPGMRRYLKDTVDKCCKNGYVETISGRRRYLPSISNKKPYVRAHAERQAVNTTVQGSAADLVKVAMNRIDDRLSAMFPLSKKTFSYKEDEVQGIELSSDRCCLVLQLHDELIYEVTERCLGQAAKVIKEEMETAMTLSVKMPVKVKSGLSWATMQDLAV

SEQ ID NO: 18 - protein, 2544 aa, M. musculus
MSLPRRSRKRRRSSSGSDTFSGDGDSFVSPQLRCGPVLSPPPGLGRGRRLTGTGTNKRRVSDDQIDQLLLANWGLPKAVLEKYHSFGVRKMFEWQAECLLLGHVLEGKNLVYSAPTSAGKTLVAELLILKRVLETRKKALFILPFVSVAKEKKCYLQSLFQEVGLKVDGYMGSTSPTGQFSSLDIAVCTIERANGLVNRLIEENKMDLLGMVVVDELHMLGDSHRGYLLELLLTKICYVTRKSASHQAESASTLSNAVQIVGMSATLPNLQLVASWLNAELYHTDFRPVPLLESIKIGNSIYDSSMKLVREFQPLLQVKGDEDHIVSLCYETIQDNHSVLIFCPSKKWCEKVADIIAREFYNLHHQPEGLVKSSEFPPVILDQKSLLEVMDQLKRSPSGLDSVLKNTVPWGVAFHHAGLTFEERDIIEGAFRQGFIRVLAATSTLSSGVNLPARRVIIRTPIFSGQPLDILTYKQMVGRAGRKGVDTMGESILVCKNSEKSKGIALLQGSLEPVHSCLQRQGEVTASMIRAILEIIVGGVASTSQDMQTYAACTFLAAAIQEGKQGMQRNQDDAQLGAIDACVTWLLENEFIQVAEPGDGTGGKVYHPTHLGSATLSSSLSPTDTLDIFADLQRAMKGFVLENDLHIVYLVTPVFEDWISIDWYRFFCLWEKLPTSMKRVAELVGVEEGFLARCVKGKVVARTERQHRQMAIHKRFFTSLVLLDLISEIPLKDINQKYGCNRGQIQSLQQSAAVYAGMITVFSNRLGWHNMELLLSQFQKRLTFGIQRELCDLIRVSLLNAQRARFLYASGFLTVADLARADSAEVEVALKNSLPFKSARKAVDEEEEAAEERRSMRTIWVTGKGLSAREAAALIVEEAKMILQQDLIEMGVRWDPKSPLSSSTHSRTSTSEVKEHTFKSQTKSSHKRLASMGRNSIRASGSNDKPSPDAERGIDDCSEHADSLCKFQGNFEPQTPSICTARKRTSLGINKEMLRKSLKEGKPSTKEVLQTFSSEKTRKTALSFSSEQVNNTLPSGRDRKYQKKSWGSSPVRDSGMHRGDLQGQTMCTSALCEDSQKSLEEQNAEFRSPGLFAKHLPSCAKEKCKKPSLPLQRQQACSRRSTESCAAVGHPAAGSSPAAARDRRGLAARETEKGNEALTENGGESQLQDTYPVSQYLEYHSEKHTNTCTRQKTLTEGQAGSSYVARDSNDAAPIKCERMKLNSKDRDSNPCRQALGSYTGRTEALQSTAKLGQAGGQCENLLNSSGVQGKTGAHATNRTEHSHASNPAFCDFGDSLDLDTQSEEIIEQMATENTMQGAKAVVIMEEGSAMQNKCHSTPGDQHVPGAANTDHVDSKKVESVKANTEKNINRGAPVSLIFHTQGENGACFKGNEHSVTDSQLNSFLQGFETQEIVKPIIPLAPQMRTPTGVEEESLPETSLNMSDSILFDSFGEDGFGQGQSPDIKANQPLLSEMTPNHFSNPPHPQEDPVMTPTVSEPQGTQQQGVCLSGESIIFSDIDSAQVIEALDNMAAFHVQENCNSVALKTLEPSDSAVLGNECPQGKLVRGDQNEGSPKPKLTETNQDNSFTWSGASFNLSPELQRILDKVSSPRENEKPKMIHVNLSSFEGNSKESHEREEINSDLGTVQRTSVFPSNEVKNRTEGLESKARHGGASSPLPRKESAAADDNGLIPPTPVPASASKVAFPEILGTSVKRQKASSALQPGESCLFGSPSDNQNQDLSQELRDSLKDYDGSVADTSFFLQSQDGLLLTQASCSSESLAIIDVASDQILFQTFVKEWQCQKRFSISLACEKMTSSMSSKTATIGGKLKQVSLPQEATVEDAGFPVRGCDGAVVVGLAVCWGAKDAYYLSLQKEQKQSEISPSLAPPPLDATLTVKERMECLQSCLQKKSDRERSVVTYDFIQTYKVLLLSCGISLEPSYEDPKVACWLLDPDSKEPTLHSIVTSFLPHELALLEGMETGPGIQSLGLNVNTEHSGRYRASVESVLIFNSMNQLNSLLQKENLHDIFCKVEMPSQYCLALLELNGIGFSTAECESQKHVMQAKLDAIETQAYQLAGHSFSFTSADDIAQVLFLELKLPPNGEMKTQGSKKTLGSTRRGNESGRRMRLGRQFSTSKDILNKLKGLHPLPGLILEWRRISNAITKVVFPLQREKHLNPLLRMERIYPVSQSHTATGRITFTEPNIQNVPRDFEIKMPTLVRESPPSQAPKGRFPMAIGQDKKVYGLHPGHRTQMEEKASDRGVPFSVSMRHAFVPFPGGLILAADYSQLELRILAHLSRDCRLIQVLNTGADVFRSIAAEWKMIEPDAVGDDLRQHAKQICYGIIYGMGAKSLGEQMGIKENDAASYIDSFKSRYKGINHFMRDTVKNCRKNGFVETILGRRRYLPGIKDDNPYHKAHAERQAINTTVQGSAADIVKIATVNIQKQLETFRSTFKSHGHRESMLQNDRTGLLPKRKLKGMFCPMRGGFFILQLHDELLYEVAEEDVVQVAQIVKNEMECAIKLSVKLKVKVKIGASWGELKDFDV

SEQ ID NO: 19 - DNA, 2397 bp, artificial sequence
  sequence of example 1
ggcttcaaggacaatagtccgatcagtgacacttctttcagtttacagctgtcacaagacggccttcaattaacacctgcctccagctcatccgaaagcctttcgatcattgacgtcgcctcggatcaaaatttgttccagacctttattaaagaatggcgttgcaaaaaacgcttcagtatttcgttggcgtgtgaaaagatccgctctcttacgtccagtaagacagcgacaatcggttcgcgcttcaagcaggccagctcaccccaagagattcccatccgcgacgacggttttcctatcaaagggtgtgatgacactttggtggtgggtctggcagtttgctggggaggacgtgatgcgtattacttcagcttgcagaaagaacaaaaacactccgaaatctctgcgtccttggtccccccttcattggacccatcattaacgcttaaagatcgtatgtggtacttgcagagttgtttacgcaaagaaagcgacaaagaatgtagtgtggtcatctatgatttcatccagagctacaaaatcttgttgttatcctgtggcatctctctggagcagagctatgaagatccgaaggtagcctgttggcttttggacccggattcgcaagagccaaccctgcattcaatcgtcaccagcttccttccacatgaactgcctcttttagagggaatggagacctcgcagggaatccaatctcttggacttaatgctggatctgaacacagtggacgctatcgcgcgtcagttgaatcaatcctgatttttaactcgatgaatcaacttaattccctgcttcagaaagaaaaccttcaggacgtctttcgtaaggtggaaatgccttcgcaatattgcttagccttattagagttgaatggaatcggattttccactgcagagtgtgagtcccagaaacatatcatgcaggccaaactggatgcaatcgagacacaagcttaccagcttgcgggtcatagcttcagcttcacatcctccgacgatatcgccgaagtcttgtttttggaattaaagctgcctcctaatcgcgagatgaagaatcaaggctccaagaagacattaggttcaacccgccgtggaatcgacaatggtcgtaaattacgtctgggccgccagtttagcacatctaaagacgtccttaataagctgaaagccttgcaccctcttccgggcctgattttggagtggcgccgtattacaaatgccatcaccaaagtagttttcccattgcagcgcgagaagtgtcttaatccattccttgggatggagcgtatctatcccgtcagccagtcacatactgcaacgggacgcattactttcacggagccaaacatccaaaatgtcccccgcgacttcgagattaaaatgcctactctggttggggagtctcctcctagccaagctgtgggcaagggactgctgcctatgggtcgtggcaaatacaaaaagggctttagtgttaacccacgctgccaggctcagatggaggagcgcgctgcagatcgtggaatgcctttttctatcagcatgcgtcacgcattcgtccccttcccagggggaagtatcttagcggctgattactctcaattggaacttcgtattctggcgcaccttagtcatgaccgtcgcttgattcaggtactgaatactggagcggacgtgtttcgttcgattgctgcggagtggaaaatgatcgagcccgaatccgtcggtgatgatcttcgtcaacaggcaaaacagatctgttacgggatcatctatggaatgggtgctaaatccttgggtgagcaaatggggattaaggagaacgatgccgcatgctacattgatagcttcaaatcacgttacaccggtattaatcaatttatgactgagaccgtgaaaaactgtaaacgtgacggcttcgtccaaacaattttagggcgtcgccgctatttaccgggaattaaggacaacaatccctaccgcaaagcacatgccgaacgtcaagcaatcaacactattgtccaaggttcggctgctgatatcgtgaaaattgccacagtcaacatccagaaacagctggagacgtttcattcaacatttaaaagccacggacaccgtgaaggcatgctgcaatcggaccaaactggtctgtcacgtaagcgtaaattgcagggtatgttctgtccgattcgcggaggcttctttatcttacaattacacgacgagctgttgtatgaagttgccgaggaagatgtcgtccaggtggctcagattgttaagaacgaaatggaatctgctgtgaagttgtctgtgaagcttaaagtcaaagttaaaattggtgcttcgtggggggagttgaaagacttcgatgtt